European Patent Application EP 4 335 925 A2, published March 13, 2024. Title: LONG-LASTING ANALGESIA VIA TARGETED IN VIVO EPIGENETIC REPRESSION. Applicant: The Regents of the University of California. Application EP. The sequence listing filed with the application follows.

SEQUENCE LISTING (143 sequences)

SEQ ID NO: 1 - DNA, 4164 bp, synthetic construct
  misc_feature 1..4164: note = dCas9
  source 1..4164: mol_type = other DNA
  CDS 1..4164
atgggccccaagaaaaaacgcaaggtggccgcagcagactataaggatgacgacgataaggggatccatggtgtgcctgctgcagataaaaaatacagcatcggcctggctatcggaactaactccgtcggctgggccgtcattaccgacgaatacaaagtacctagcaaaaagttcaaggtgcttggcaacacagatcgccactcaatcaagaaaaaccttatcggagccctgctgtttgactcaggcgaaaccgccgaggctacacgcctgaaaagaacagctagacggcggtacaccagaaggaagaaccggatctgttatcttcaggagattttctccaatgagatggctaaggtggacgattctttcttccatcgactcgaagaatctttcttggtggaggaagataagaaacacgagaggcatcctattttcggaaacattgtcgatgaagtggcctatcatgagaaataccccacgatctaccatctgcgaaaaaagttggttgactctaccgacaaggcggacctgaggcttatttatctggccctggcccatatgatcaaattcagggggcacttcttgatcgagggggaccttaatcccgacaactctgacgtggataagttgttcatacagcttgtgcagacctacaaccagctgttcgaggagaatccaatcaacgccagcggagtggacgctaaagccattctgagcgcgagattgagcaagtctagaagattggaaaaccttatagcccagctgccaggtgagaagaagaacggactgtttggcaatctcattgcgcttagcctcggactcaccccgaacttcaaatccaacttcgacctcgccgaagatgccaaattgcagctcagtaaggatacgtatgacgatgatcttgacaatctgctggcgcagatcggggaccagtacgccgatcttttcttggcagcaaaaaatctctcagatgcaatactcttgtcagacatactgcgagttaataccgagattactaaggctccgctttctgcctccatgatcaagcgctacgatgagcatcaccaggatctgacactgttgaaagccctggtgcgccaacagctgccagagaaatacaaggaaatcttttttgaccagtccaagaatggctacgcaggatacatcgatggaggagccagtcaggaggaattttacaagtttattaagcctatcctggagaagatggatggtaccgaagaactcctggtcaagctcaaccgagaagatttgcttcgcaagcaaaggacttttgacaacggctccattccgcatcagattcatctgggcgagctgcatgccattctgcgaagacaggaggatttttacccatttctgaaggacaaccgagagaagatcgagaaaatactgacattcaggataccatattacgtgggtccactcgccaggggcaactcccgattcgcctggatgacaaggaaaagcgaagagacgatcactccatggaacttcgaggaggtcgtggacaagggggcctccgcgcagagctttatcgagaggatgacgaactttgacaaaaatctccctaacgagaaggtgctgccaaaacattctctgctctacgagtatttcaccgtttataatgagctcacaaaggtgaagtacgtgaccgaagggtgcttcgacagcgttgagatttccggcgtggaggatagattcaacgcttctctcggcacttatcacgaccttctgaagattatcaaggataaggatttcctggacaacgaagagaatgaagacatcctggaggacatcgtcctgaccttgaccctgttcgaggacagagagatgatcgaggagaggcttaagacctacgcccacctgtttgatgacaaagtgatgaaacagctgaaacggagacggtatactggttggggcaggctgtcccggaagcttattaacggaatacgggataagcaaagtggaaagacaatacttgacttcctgaagtctgatggttttgctaacaggaatttcatgcagctgattcacgacgactcccttacatttaaggaggacattcagaaggcccaggtgtctggacaaggggactctctccatgagcacatcgccaacctggccggcagcccagccatcaaaaaaggaattcttcaaactgtaaaggtggtggatgagctggttaaagtcatgggacggcacaagcctgagaatatcgtcattgagatggccagggagaatcagacgacacagaaaggacagaagaactcacgcgagaggatgaagagaattgaggaagggataaaggagctgggaagtcagattctgaaggaacacccagttgaaaatacccagctgcagaatgaaaagctgtatctgtactatctgcagaatggacgagacatgtatgttgatcaggagctggacattaaccgactctcagattatgacgtggatgctatagtccctcagagtttcctcaaggacgattcaatcgataataaagtgttgacccgcagcgacaaaaacaggggcaaaagcgataatgtgccctcagaggaagtggtcaagaaaatgaagaattactggagacagctgctcaacgctaagcttattacccagaggaaattcgataatttgacaaaagctgaaaggggtgggcttagcgagctggataaagcaggattcatcaagcggcagcttgtcgagacgcgccagatcacaaagcacgtggcacagattttggattcccgcatgaacactaagtatgacgagaacgataagctgatccgcgaggtgaaggtgatcacgctgaagtccaagctggtaagtgatttccggaaagatttccagttctacaaagtgagggagattaacaactatcaccacgcccacgacgcttacttgaatgccgttgtgggtacagcattgatcaaaaaatatccaaagctggaaagtgagtttgtttacggagactataaagtctatgacgtgcggaagatgatcgccaagagcgagcaggagatcgggaaagcaacagctaaatatttcttctattccaatatcatgaattttttcaaaactgagataacacttgctaatggtgagataagaaagcgaccgctgatagagacgaatggcgagactggcgagatcgtgtgggacaaagggagggacttcgcaaccgtccgcaaggtcttgagcatgccgcaggtgaatatagttaagaaaaccgaagtgcaaacaggcggcttcagtaaggagtccatattgccgaagaggaactctgacaagctgatcgctaggaaaaaggattgggatccaaaaaaatacggcgggttcgactcccctaccgttgcatacagcgtgcttgtggtcgcgaaggtcgaaaagggcaagtctaagaagctcaagagtgtcaaagaattgctgggtatcacaattatggagcgcagtagtttcgagaagaatccgatagattttctggaggcaaagggatacaaggaggtgaagaaggatctgatcatcaaactgcctaagtactccctgttcgagcttgagaatggtagaaagcgcatgcttgcctcagccggcgaattgcagaagggcaatgagctcgccctgccttcaaaatacgtgaacttcctgtacttggcatcacactacgaaaagctgaaaggatcccctgaggataatgagcaaaaacaactttttgtggagcagcataagcactatctcgatgaaattattgagcagatttctgaattcagcaagcgcgtcatcctcgcggacgccaatctggataaagtgctgagcgcctacaataaacaccgagacaagcccattcgggaacaggccgagaacatcattcacctcttcactctgactaatctcggggccccggccgcattcaaatacttcgacactactatcgacaggaaacgctatacttcaacgaaggaggtgctggacgctactttgatccaccagtccattacggggctctatgagacacgaatcgatctttctcaacttggaggtgatgcctacccatatgacgtgcctgactatgcctccctgggctctgggagccctaagaaaaagaggaaggtagaggatccaaaaaaaaagcgaaaagtcgat

SEQ ID NO: 2 - protein, 1388 aa, synthetic construct
  REGION 1..1388: note = Synthetic Construct
MGPKKKRKVAAADYKDDDDKGIHGVPAADKKYSIGLAIGTNSVGWAVITDEYKVPSKKFKVLGNTDRHSIKKNLIGALLFDSGETAEATRLKRTARRRYTRRKNRICYLQEIFSNEMAKVDDSFFHRLEESFLVEEDKKHERHPIFGNIVDEVAYHEKYPTIYHLRKKLVDSTDKADLRLIYLALAHMIKFRGHFLIEGDLNPDNSDVDKLFIQLVQTYNQLFEENPINASGVDAKAILSARLSKSRRLENLIAQLPGEKKNGLFGNLIALSLGLTPNFKSNFDLAEDAKLQLSKDTYDDDLDNLLAQIGDQYADLFLAAKNLSDAILLSDILRVNTEITKAPLSASMIKRYDEHHQDLTLLKALVRQQLPEKYKEIFFDQSKNGYAGYIDGGASQEEFYKFIKPILEKMDGTEELLVKLNREDLLRKQRTFDNGSIPHQIHLGELHAILRRQEDFYPFLKDNREKIEKILTFRIPYYVGPLARGNSRFAWMTRKSEETITPWNFEEVVDKGASAQSFIERMTNFDKNLPNEKVLPKHSLLYEYFTVYNELTKVKYVTEGCFDSVEISGVEDRFNASLGTYHDLLKIIKDKDFLDNEENEDILEDIVLTLTLFEDREMIEERLKTYAHLFDDKVMKQLKRRRYTGWGRLSRKLINGIRDKQSGKTILDFLKSDGFANRNFMQLIHDDSLTFKEDIQKAQVSGQGDSLHEHIANLAGSPAIKKGILQTVKVVDELVKVMGRHKPENIVIEMARENQTTQKGQKNSRERMKRIEEGIKELGSQILKEHPVENTQLQNEKLYLYYLQNGRDMYVDQELDINRLSDYDVDAIVPQSFLKDDSIDNKVLTRSDKNRGKSDNVPSEEVVKKMKNYWRQLLNAKLITQRKFDNLTKAERGGLSELDKAGFIKRQLVETRQITKHVAQILDSRMNTKYDENDKLIREVKVITLKSKLVSDFRKDFQFYKVREINNYHHAHDAYLNAVVGTALIKKYPKLESEFVYGDYKVYDVRKMIAKSEQEIGKATAKYFFYSNIMNFFKTEITLANGEIRKRPLIETNGETGEIVWDKGRDFATVRKVLSMPQVNIVKKTEVQTGGFSKESILPKRNSDKLIARKKDWDPKKYGGFDSPTVAYSVLVVAKVEKGKSKKLKSVKELLGITIMERSSFEKNPIDFLEAKGYKEVKKDLIIKLPKYSLFELENGRKRMLASAGELQKGNELALPSKYVNFLYLASHYEKLKGSPEDNEQKQLFVEQHKHYLDEIIEQISEFSKRVILADANLDKVLSAYNKHRDKPIREQAENIIHLFTLTNLGAPAAFKYFDTTIDRKRYTSTKEVLDATLIHQSITGLYETRIDLSQLGGDAYPYDVPDYASLGSGSPKKKRKVEDPKKKRKVD

SEQ ID NO: 3 - DNA, 7256 bp, synthetic construct
  misc_feature 1..7256: note = AAV, dNCas9
  source 1..7256: mol_type = other DNA
ctgcgcgctcgctcgctcactgaggccgcccgggcaaagcccgggcgtcgggcgacctttggtcgcccggcctcagtgagcgagcgagcgcgcagagagggagtggccaactccatcactaggggttccttgtagttaatgattaacccgccatgctacttatctacgtagccatgctctaggaagatcggaattcgcccttaagctagctagttattaatagtaatcaattacggggtcattagttcatagcccatatatggagttccgcgttacataacttacggtaaatggcccgcctggctgaccgcccaacgacccccgcccattgacgtcaataatgacgtatgttcccatagtaacgccaatagggactttccattgacgtcaatgggtggagtatttacggtaaactgcccacttggcagtacatcaagtgtatcatatgccaagtacgccccctattgacgtcaatgacggtaaatggcccgcctggcattatgcccagtacatgaccttatgggactttcctacttggcagtacatctacgtattagtcatcgctattaccatggtgatgcggttttggcagtacatcaatgggcgtggatagcggtttgactcacggggatttccaagtctccaccccattgacgtcaatgggagtttgttttggcaccaaaatcaacgggactttccaaaatgtcgtaacaactccgccccattgacgcaaatgggcggtaggcgtgtacggtgggaggtctatataagcagagctggtttagtgaaccgtcagatcctgcagaagttggtcgtgaggcactgggcaggtaagtatcaaggttacaagacaggtttaaggagaccaatagaaactgggcttgtcgagacagagaagactcttgcgtttctgataggcacctattggtcttactgacatccactttgcctttctctccacaggtgtccaggcggccgccatggatatcatcatgggccccaagaaaaaacgcaaggtggccgcagcagactataaggatgacgacgataaggggatccatggtgtgcctgctgcagataaaaaatacagcatcggcctggctatcggaactaactccgtcggctgggccgtcattaccgacgaatacaaagtacctagcaaaaagttcaaggtgcttggcaacacagatcgccactcaatcaagaaaaaccttatcggagccctgctgtttgactcaggcgaaaccgccgaggctacacgcctgaaaagaacagctagacggcggtacaccagaaggaagaaccggatctgttatcttcaggagattttctccaatgagatggctaaggtggacgattctttcttccatcgactcgaagaatctttcttggtggaggaagataagaaacacgagaggcatcctattttcggaaacattgtcgatgaagtggcctatcatgagaaataccccacgatctaccatctgcgaaaaaagttggttgactctaccgacaaggcggacctgaggcttatttatctggccctggcccatatgatcaaattcagggggcacttcttgatcgagggggaccttaatcccgacaactctgacgtggataagttgttcatacagcttgtgcagacctacaaccagctgttcgaggagaatccaatcaacgccagcggagtggacgctaaagccattctgagcgcgagattgagcaagtctagaagattggaaaaccttatagcccagctgccaggtgagaagaagaacggactgtttggcaatctcattgcgcttagcctcggactcaccccgaacttcaaatccaacttcgacctcgccgaagatgccaaattgcagctcagtaaggatacgtatgacgatgatcttgacaatctgctggcgcagatcggggaccagtacgccgatcttttcttggcagcaaaaaatctctcagatgcaatactcttgtcagacatactgcgagttaataccgagattactaaggctccgctttctgcctccatgatcaagcgctacgatgagcatcaccaggatctgacactgttgaaagccctggtgcgccaacagctgccagagaaatacaaggaaatcttttttgaccagtccaagaatggctacgcaggatacatcgatggaggagccagtcaggaggaattttacaagtttattaagcctatcctggagaagatggatggtaccgaagaactcctggtcaagctcaaccgagaagatttgcttcgcaagcaaaggacttttgacaacggctccattccgcatcagattcatctgggcgagctgcatgccattctgcgaagacaggaggatttttacccatttctgaaggacaaccgagagaagatcgagaaaatactgacattcaggataccatattacgtgggtccactcgccaggggcaactcccgattcgcctggatgacaaggaaaagcgaagagacgatcactccatggaacttcgaggaggtcgtggacaagggggcctccgcgcagagctttatcgagaggatgacgaactttgacaaaaatctccctaacgagaaggtgctgccaaaacattctctgctctacgagtatttcaccgtttataatgagctcacaaaggtgaagtacgtgaccgaagggatgcggaagcccgcttttctgtccggagagcagaagaaggctatcgtggatttgctctttaagactaaccgcaaggtaacagtcaagcagctgaaggaagactacttcaagaagatcgaatgcttgtcctacgaaacggaaatcttgacagttgagtacgggctcctgccaatcgggaagatagtagagaagaggattgaatgtaccgtctattctgttgataacaacggtaacatatacacccagcccgtcgcccaatggcacgatcgcggtgagcaggaggtgttcgaatactgtctggaggacgggtcattgattcgggcgactaaggaccataagtttatgacggtagacggccagatgttgcccatagatgagatctttgagcgggaactcgacttgatgagagtcgataatcttcctaattaaaccggagcttggatccaatcaacctctggattacaaaatttgtgaaagattgactggtattcttaactatgttgctccttttacgctatgtggatacgctgctttaatgcctttgtatcatgctattgcttcccgtatggctttcattttctcctccttgtataaatcctggttgctgtctctttatgaggagttgtggcccgttgtcaggcaacgtggcgtggtgtgcactgtgtttgctgacgcaacccccactggttggggcattgccaccacctgtcagctcctttccgggactttcgctttccccctccctattgccacggcggaactcatcgccgcctgccttgcccgctgctggacaggggctcggctgttgggcactgacaattccgtggtgttgtcggggaaatcatcgtcctttccttggctgctcgcctgtgttgccacctggattctgcgcgggacgtccttctgctacgtcccttcggccctcaatccagcggaccttccttcccgcggcctgctgccggctctgcggcctcttccgcgtcttcgagatctgcctcgactgtgccttctagttgccagccatctgttgtttgcccctcccccgtgccttccttgaccctggaaggtgccactcccactgtcctttcctaataaaatgaggaaattgcatcgcattgtctgagtaggtgtcattctattctggggggtggggtggggcaggacagcaagggggaggattgggaagacaatagcaggcatgctggggactcgagacgcgtggaggagggcctatttcccatgattccttcatatttgcatatacgatacaaggctgttagagagataattagaattaatttgactgtaaacacaaagatattagtacaaaatacgtgacgtagaaagtaataatttcttgggtagtttgcagttttaaaattatgttttaaaatggactatcatatgcttaccgtaacttgaaagtatttcgatttcttggctttatatatcttgtggaaaggacgaaacaccggttttagagctagaaatagcaagttaaaataaggctagtccgttatcaacttgaaaaagtggcaccgagtcggtgcttttttctcgagttaagggcgaattcccgataaggatcttcctagagcatggctacgtagataagtagcatggcgggttaatcattaactacaaggaacccctagtgatggagttggccactccctctctgcgcgctcgctcgctcactgaggccgggcgaccaaaggtcgcccgacgcccgggctttgcccgggcggcctcagtgagcgagcgagcgcgcagccttaattaacctaattcactggccgtcgttttacaacgtcgtgactgggaaaaccctggcgttacccaacttaatcgccttgcagcacatccccctttcgccagctggcgtaatagcgaagaggcccgcaccgatcgcccttcccaacagttgcgcagcctgaatggcgaatgggacgcgccctgtagcggcgcattaagcgcggcgggtgtggtggttacgcgcagcgtgaccgctacacttgccagcgccctagcgcccgctcctttcgctttcttcccttcctttctcgccacgttcgccggctttccccgtcaagctctaaatcgggggctccctttagggttccgatttagtgctttacggcacctcgaccccaaaaaacttgattagggtgatggttcacgtagtgggccatcgccctgatagacggtttttcgccctttgacgttggagtccacgttctttaatagtggactcttgttccaaactggaacaacactcaaccctatctcggtctattcttttgatttataagggattttgccgatttcggcctattggttaaaaaatgagctgatttaacaaaaatttaacgcgaattttaacaaaatattaacgtttataatttcaggtggcatctttcggggaaatgtgcgcggaacccctatttgtttatttttctaaatacattcaaatatgtatccgctcatgagacaataaccctgataaatgcttcaataatattgaaaaaggaagagtatgagtattcaacatttccgtgtcgcccttattcccttttttgcggcattttgccttcctgtttttgctcacccagaaacgctggtgaaagtaaaagatgctgaagatcagttgggtgcacgagtgggttacatcgaactggatctcaatagtggtaagatccttgagagttttcgccccgaagaacgttttccaatgatgagcacttttaaagttctgctatgtggcgcggtattatcccgtattgacgccgggcaagagcaactcggtcgccgcatacactattctcagaatgacttggttgagtactcaccagtcacagaaaagcatcttacggatggcatgacagtaagagaattatgcagtgctgccataaccatgagtgataacactgcggccaacttacttctgacaacgatcggaggaccgaaggagctaaccgcttttttgcacaacatgggggatcatgtaactcgccttgatcgttgggaaccggagctgaatgaagccataccaaacgacgagcgtgacaccacgatgcctgtagtaatggtaacaacgttgcgcaaactattaactggcgaactacttactctagcttcccggcaacaattaatagactggatggaggcggataaagttgcaggaccacttctgcgctcggcccttccggctggctggtttattgctgataaatctggagccggtgagcgtgggtctcgcggtatcattgcagcactggggccagatggtaagccctcccgtatcgtagttatctacacgacggggagtcaggcaactatggatgaacgaaatagacagatcgctgagataggtgcctcactgattaagcattggtaactgtcagaccaagtttactcatatatactttagattgatttaaaacttcatttttaatttaaaaggatctaggtgaagatcctttttgataatctcatgaccaaaatcccttaacgtgagttttcgttccactgagcgtcagaccccgtagaaaagatcaaaggatcttcttgagatcctttttttctgcgcgtaatctgctgcttgcaaacaaaaaaaccaccgctaccagcggtggtttgtttgccggatcaagagctaccaactctttttccgaaggtaactggcttcagcagagcgcagataccaaatactgtccttctagtgtagccgtagttaggccaccacttcaagaactctgtagcaccgcctacatacctcgctctgctaatcctgttaccagtggctgctgccagtggcgataagtcgtgtcttaccgggttggactcaagacgatagttaccggataaggcgcagcggtcgggctgaacggggggttcgtgcacacagcccagcttggagcgaacgacctacaccgaactgagatacctacagcgtgagctatgagaaagcgccacgcttcccgaagggagaaaggcggacaggtatccggtaagcggcagggtcggaacaggagagcgcacgagggagcttccagggggaaacgcctggtatctttatagtcctgtcgggtttcgccacctctgacttgagcgtcgatttttgtgatgctcgtcaggggggcggagcctatggaaaaacgccagcaacgcggcctttttacggttcctggccttttgctgcggttttgctcacatgttctttcctgcgttatcccctgattctgtggataaccgtattaccgcctttgagtgagctgataccgctcgccgcagccgaacgaccgagcgcagcgagtcagtgagcgaggaagcggaagagcgcccaatacgcaaaccgcctctccccgcgcgttggccgattcattaatgcagctggcacgacaggtttcccgactggaaagcgggcagtgagcgcaacgcaattaatgtgagttagctcactcattaggcaccccaggctttacactttatgcttccggctcgtatgttgtgtggaattgtgagcggataacaatttcacacaggaaacagctatgaccatgattacgccagatttaattaagg

SEQ ID NO: 4 - DNA, 7736 bp, synthetic construct
  misc_feature 1..7736: note = AAV, dCCas9
  source 1..7736: mol_type = other DNA
ctgcgcgctcgctcgctcactgaggccgcccgggcaaagcccgggcgtcgggcgacctttggtcgcccggcctcagtgagcgagcgagcgcgcagagagggagtggccaactccatcactaggggttccttgtagttaatgattaacccgccatgctacttatctacgtagccatgctctaggaagatcggaattcgcccttaagctagctagttattaatagtaatcaattacggggtcattagttcatagcccatatatggagttccgcgttacataacttacggtaaatggcccgcctggctgaccgcccaacgacccccgcccattgacgtcaataatgacgtatgttcccatagtaacgccaatagggactttccattgacgtcaatgggtggagtatttacggtaaactgcccacttggcagtacatcaagtgtatcatatgccaagtacgccccctattgacgtcaatgacggtaaatggcccgcctggcattatgcccagtacatgaccttatgggactttcctacttggcagtacatctacgtattagtcatcgctattaccatggtgatgcggttttggcagtacatcaatgggcgtggatagcggtttgactcacggggatttccaagtctccaccccattgacgtcaatgggagtttgttttggcaccaaaatcaacgggactttccaaaatgtcgtaacaactccgccccattgacgcaaatgggcggtaggcgtgtacggtgggaggtctatataagcagagctggtttagtgaaccgtcagatcctgcagaagttggtcgtgaggcactgggcaggtaagtatcaaggttacaagacaggtttaaggagaccaatagaaactgggcttgtcgagacagagaagactcttgcgtttctgataggcacctattggtcttactgacatccactttgcctttctctccacaggtgtccaggcggccgccatggatatcatgattaagatcgcaacccgaaaatacctgggaaagcagaacgtctacgatattggtgtagagagagaccataactttgctctgaagaacggctttattgcctcatgcttcgacagcgttgagatttccggcgtggaggatagattcaacgcttctctcggcacttatcacgaccttctgaagattatcaaggataaggatttcctggacaacgaagagaatgaagacatcctggaggacatcgtcctgaccttgaccctgttcgaggacagagagatgatcgaggagaggcttaagacctacgcccacctgtttgatgacaaagtgatgaaacagctgaaacggagacggtatactggttggggcaggctgtcccggaagcttattaacggaatacgggataagcaaagtggaaagacaatacttgacttcctgaagtctgatggttttgctaacaggaatttcatgcagctgattcacgacgactcccttacatttaaggaggacattcagaaggcccaggtgtctggacaaggggactctctccatgagcacatcgccaacctggccggcagcccagccatcaaaaaaggaattcttcaaactgtaaaggtggtggatgagctggttaaagtcatgggacggcacaagcctgagaatatcgtcattgagatggccagggagaatcagacgacacagaaaggacagaagaactcacgcgagaggatgaagagaattgaggaagggataaaggagctgggaagtcagattctgaaggaacacccagttgaaaatacccagctgcagaatgaaaagctgtatctgtactatctgcagaatggacgagacatgtatgttgatcaggagctggacattaaccgactctcagattatgacgtggatgctatagtccctcagagtttcctcaaggacgattcaatcgataataaagtgttgacccgcagcgacaaaaacaggggcaaaagcgataatgtgccctcagaggaagtggtcaagaaaatgaagaattactggagacagctgctcaacgctaagcttattacccagaggaaattcgataatttgacaaaagctgaaaggggtgggcttagcgagctggataaagcaggattcatcaagcggcagcttgtcgagacgcgccagatcacaaagcacgtggcacagattttggattcccgcatgaacactaagtatgacgagaacgataagctgatccgcgaggtgaaggtgatcacgctgaagtccaagctggtaagtgatttccggaaagatttccagttctacaaagtgagggagattaacaactatcaccacgcccacgacgcttacttgaatgccgttgtgggtacagcattgatcaaaaaatatccaaagctggaaagtgagtttgtttacggagactataaagtctatgacgtgcggaagatgatcgccaagagcgagcaggagatcgggaaagcaacagctaaatatttcttctattccaatatcatgaattttttcaaaactgagataacacttgctaatggtgagataagaaagcgaccgctgatagagacgaatggcgagactggcgagatcgtgtgggacaaagggagggacttcgcaaccgtccgcaaggtcttgagcatgccgcaggtgaatatagttaagaaaaccgaagtgcaaacaggcggcttcagtaaggagtccatattgccgaagaggaactctgacaagctgatcgctaggaaaaaggattgggatccaaaaaaatacggcgggttcgactcccctaccgttgcatacagcgtgcttgtggtcgcgaaggtcgaaaagggcaagtctaagaagctcaagagtgtcaaagaattgctgggtatcacaattatggagcgcagtagtttcgagaagaatccgatagattttctggaggcaaagggatacaaggaggtgaagaaggatctgatcatcaaactgcctaagtactccctgttcgagcttgagaatggtagaaagcgcatgcttgcctcagccggcgaattgcagaagggcaatgagctcgccctgccttcaaaatacgtgaacttcctgtacttggcatcacactacgaaaagctgaaaggatcccctgaggataatgagcaaaaacaactttttgtggagcagcataagcactatctcgatgaaattattgagcagatttctgaattcagcaagcgcgtcatcctcgcggacgccaatctggataaagtgctgagcgcctacaataaacaccgagacaagcccattcgggaacaggccgagaacatcattcacctcttcactctgactaatctcggggccccggccgcattcaaatacttcgacactactatcgacaggaaacgctatacttcaacgaaggaggtgctggacgctactttgatccaccagtccattacggggctctatgagacacgaatcgatctttctcaacttggaggtgatgcctacccatatgacgtgcctgactatgcctccctgggctctgggagccctaagaaaaagaggaaggtagaggatccaaaaaaaaagcgaaaagtcgattaaaccggagcttggatccaatcaacctctggattacaaaatttgtgaaagattgactggtattcttaactatgttgctccttttacgctatgtggatacgctgctttaatgcctttgtatcatgctattgcttcccgtatggctttcattttctcctccttgtataaatcctggttgctgtctctttatgaggagttgtggcccgttgtcaggcaacgtggcgtggtgtgcactgtgtttgctgacgcaacccccactggttggggcattgccaccacctgtcagctcctttccgggactttcgctttccccctccctattgccacggcggaactcatcgccgcctgccttgcccgctgctggacaggggctcggctgttgggcactgacaattccgtggtgttgtcggggaaatcatcgtcctttccttggctgctcgcctgtgttgccacctggattctgcgcgggacgtccttctgctacgtcccttcggccctcaatccagcggaccttccttcccgcggcctgctgccggctctgcggcctcttccgcgtcttcgagatctgcctcgactgtgccttctagttgccagccatctgttgtttgcccctcccccgtgccttccttgaccctggaaggtgccactcccactgtcctttcctaataaaatgaggaaattgcatcgcattgtctgagtaggtgtcattctattctggggggtggggtggggcaggacagcaagggggaggattgggaagacaatagcaggcatgctggggactcgagacgcgtggaggagggcctatttcccatgattccttcatatttgcatatacgatacaaggctgttagagagataattagaattaatttgactgtaaacacaaagatattagtacaaaatacgtgacgtagaaagtaataatttcttgggtagtttgcagttttaaaattatgttttaaaatggactatcatatgcttaccgtaacttgaaagtatttcgatttcttggctttatatatcttgtggaaaggacgaaacaccggttttagagctagaaatagcaagttaaaataaggctagtccgttatcaacttgaaaaagtggcaccgagtcggtgcttttttctcgagttaagggcgaattcccgataaggatcttcctagagcatggctacgtagataagtagcatggcgggttaatcattaactacaaggaacccctagtgatggagttggccactccctctctgcgcgctcgctcgctcactgaggccgggcgaccaaaggtcgcccgacgcccgggctttgcccgggcggcctcagtgagcgagcgagcgcgcagccttaattaacctaattcactggccgtcgttttacaacgtcgtgactgggaaaaccctggcgttacccaacttaatcgccttgcagcacatccccctttcgccagctggcgtaatagcgaagaggcccgcaccgatcgcccttcccaacagttgcgcagcctgaatggcgaatgggacgcgccctgtagcggcgcattaagcgcggcgggtgtggtggttacgcgcagcgtgaccgctacacttgccagcgccctagcgcccgctcctttcgctttcttcccttcctttctcgccacgttcgccggctttccccgtcaagctctaaatcgggggctccctttagggttccgatttagtgctttacggcacctcgaccccaaaaaacttgattagggtgatggttcacgtagtgggccatcgccctgatagacggtttttcgccctttgacgttggagtccacgttctttaatagtggactcttgttccaaactggaacaacactcaaccctatctcggtctattcttttgatttataagggattttgccgatttcggcctattggttaaaaaatgagctgatttaacaaaaatttaacgcgaattttaacaaaatattaacgtttataatttcaggtggcatctttcggggaaatgtgcgcggaacccctatttgtttatttttctaaatacattcaaatatgtatccgctcatgagacaataaccctgataaatgcttcaataatattgaaaaaggaagagtatgagtattcaacatttccgtgtcgcccttattcccttttttgcggcattttgccttcctgtttttgctcacccagaaacgctggtgaaagtaaaagatgctgaagatcagttgggtgcacgagtgggttacatcgaactggatctcaatagtggtaagatccttgagagttttcgccccgaagaacgttttccaatgatgagcacttttaaagttctgctatgtggcgcggtattatcccgtattgacgccgggcaagagcaactcggtcgccgcatacactattctcagaatgacttggttgagtactcaccagtcacagaaaagcatcttacggatggcatgacagtaagagaattatgcagtgctgccataaccatgagtgataacactgcggccaacttacttctgacaacgatcggaggaccgaaggagctaaccgcttttttgcacaacatgggggatcatgtaactcgccttgatcgttgggaaccggagctgaatgaagccataccaaacgacgagcgtgacaccacgatgcctgtagtaatggtaacaacgttgcgcaaactattaactggcgaactacttactctagcttcccggcaacaattaatagactggatggaggcggataaagttgcaggaccacttctgcgctcggcccttccggctggctggtttattgctgataaatctggagccggtgagcgtgggtctcgcggtatcattgcagcactggggccagatggtaagccctcccgtatcgtagttatctacacgacggggagtcaggcaactatggatgaacgaaatagacagatcgctgagataggtgcctcactgattaagcattggtaactgtcagaccaagtttactcatatatactttagattgatttaaaacttcatttttaatttaaaaggatctaggtgaagatcctttttgataatctcatgaccaaaatcccttaacgtgagttttcgttccactgagcgtcagaccccgtagaaaagatcaaaggatcttcttgagatcctttttttctgcgcgtaatctgctgcttgcaaacaaaaaaaccaccgctaccagcggtggtttgtttgccggatcaagagctaccaactctttttccgaaggtaactggcttcagcagagcgcagataccaaatactgtccttctagtgtagccgtagttaggccaccacttcaagaactctgtagcaccgcctacatacctcgctctgctaatcctgttaccagtggctgctgccagtggcgataagtcgtgtcttaccgggttggactcaagacgatagttaccggataaggcgcagcggtcgggctgaacggggggttcgtgcacacagcccagcttggagcgaacgacctacaccgaactgagatacctacagcgtgagctatgagaaagcgccacgcttcccgaagggagaaaggcggacaggtatccggtaagcggcagggtcggaacaggagagcgcacgagggagcttccagggggaaacgcctggtatctttatagtcctgtcgggtttcgccacctctgacttgagcgtcgatttttgtgatgctcgtcaggggggcggagcctatggaaaaacgccagcaacgcggcctttttacggttcctggccttttgctgcggttttgctcacatgttctttcctgcgttatcccctgattctgtggataaccgtattaccgcctttgagtgagctgataccgctcgccgcagccgaacgaccgagcgcagcgagtcagtgagcgaggaagcggaagagcgcccaatacgcaaaccgcctctccccgcgcgttggccgattcattaatgcagctggcacgacaggtttcccgactggaaagcgggcagtgagcgcaacgcaattaatgtgagttagctcactcattaggcaccccaggctttacactttatgcttccggctcgtatgttgtgtggaattgtgagcggataacaatttcacacaggaaacagctatgaccatgattacgccagatttaattaagg

SEQ ID NO: 5 - DNA, 5704 bp, synthetic construct
  misc_feature 1..5704: note = AAV, ZF
  source 1..5704: mol_type = other DNA
ctgcgcgctcgctcgctcactgaggccgcccgggcaaagcccgggcgtcgggcgacctttggtcgcccggcctcagtgagcgagcgagcgcgcagagagggagtggccaactccatcactaggggttccttgtagttaatgattaacccgccatgctacttatctacgtagccatgctctaggaagatcggaattcgcccttaagctagctagttattaatagtaatcaattacggggtcattagttcatagcccatatatggagttccgcgttacataacttacggtaaatggcccgcctggctgaccgcccaacgacccccgcccattgacgtcaataatgacgtatgttcccatagtaacgccaatagggactttccattgacgtcaatgggtggagtatttacggtaaactgcccacttggcagtacatcaagtgtatcatatgccaagtacgccccctattgacgtcaatgacggtaaatggcccgcctggcattatgcccagtacatgaccttatgggactttcctacttggcagtacatctacgtattagtcatcgctattaccatggtgatgcggttttggcagtacatcaatgggcgtggatagcggtttgactcacggggatttccaagtctccaccccattgacgtcaatgggagtttgttttggcaccaaaatcaacgggactttccaaaatgtcgtaacaactccgccccattgacgcaaatgggcggtaggcgtgtacggtgggaggtctatataagcagagctggtttagtgaaccgtcagatcctgcagaagttggtcgtgaggcactgggcaggtaagtatcaaggttacaagacaggtttaaggagaccaatagaaactgggcttgtcgagacagagaagactcttgcgtttctgataggcacctattggtcttactgacatccactttgcctttctctccacaggtgtccaggcggccgccatgaggagcatgcacgattacaaagaccacgatggtgactataaagaccatgatatagactataaggacgacgacgacaaaatggcacctaaaaaaaagcgcaaggtaggcattcatggcgtacccgcggcgatggctgagaggccttttcagtgccggatctgtatgagaaacttcagtgaccgcagtcatctcaccaggcacatccgcacacacacgggggagaaacccttcgcatgtgacatttgcggccgaaagttcgccgatcgaagtcatcttgcgagacacaccaaaattcacaccgggagccaaaagccctttcaatgtcgaatttgtatgcgaaatttttcccgcagcgataatctgtctgagcatattaggacgcataccggggagaagcccttcgcatgcgatatatgtggtcggaagttcgctaggtctgccgctctggcgcggcatactaaaatacacacggggagtcaaaaaccctttcagtgccggatctgcatgcggaatttttcccgatccgatacattgtcacaacacattcggacacacacaggagaaaaacctttcgcctgtgatatttgcggacgcaagtttgccacgagggatcaccggataaaacacacgaaaatccacctgcgccaaaaagacgccgcgagagggtcacgcaccttggtgacatttaaagatgttttcgtagatttcacacgagaggaatggaaactcttggacaccgcgcaacagattgtataccggaacgttatgctggaaaactataagaacctggtctctctgggttaccagttgactaaacccgatgtcattctgagactggagaaaggcgaggagccgtggctggtggactacaaggatgacgatgacaagcggagctaaacaaattttgtaatccaggcggccgccggatccaatcaacctctggattacaaaatttgtgaaagattgactggtattcttaactatgttgctccttttacgctatgtggatacgctgctttaatgcctttgtatcatgctattgcttcccgtatggctttcattttctcctccttgtataaatcctggttgctgtctctttatgaggagttgtggcccgttgtcaggcaacgtggcgtggtgtgcactgtgtttgctgacgcaacccccactggttggggcattgccaccacctgtcagctcctttccgggactttcgctttccccctccctattgccacggcggaactcatcgccgcctgccttgcccgctgctggacaggggctcggctgttgggcactgacaattccgtggtgttgtcggggaaatcatcgtcctttccttggctgctcgcctgtgttgccacctggattctgcgcgggacgtccttctgctacgtcccttcggccctcaatccagcggaccttccttcccgcggcctgctgccggctctgcggcctcttccgcgtcttcgagatctgcctcgactgtgccttctagttgccagccatctgttgtttgcccctcccccgtgccttccttgaccctggaaggtgccactcccactgtcctttcctaataaaatgaggaaattgcatcgcattgtctgagtaggtgtcattctattctggggggtggggtggggcaggacagcaagggggaggattgggaagacaatagcaggcatgctggggactcgagttaagggcgaattcccgataaggatcttcctagagcatggctacgtagataagtagcatggcgggttaatcattaactacaaggaacccctagtgatggagttggccactccctctctgcgcgctcgctcgctcactgaggccgggcgaccaaaggtcgcccgacgcccgggctttgcccgggcggcctcagtgagcgagcgagcgcgcagccttaattaacctaattcactggccgtcgttttacaacgtcgtgactgggaaaaccctggcgttacccaacttaatcgccttgcagcacatccccctttcgccagctggcgtaatagcgaagaggcccgcaccgatcgcccttcccaacagttgcgcagcctgaatggcgaatgggacgcgccctgtagcggcgcattaagcgcggcgggtgtggtggttacgcgcagcgtgaccgctacacttgccagcgccctagcgcccgctcctttcgctttcttcccttcctttctcgccacgttcgccggctttccccgtcaagctctaaatcgggggctccctttagggttccgatttagtgctttacggcacctcgaccccaaaaaacttgattagggtgatggttcacgtagtgggccatcgccctgatagacggtttttcgccctttgacgttggagtccacgttctttaatagtggactcttgttccaaactggaacaacactcaaccctatctcggtctattcttttgatttataagggattttgccgatttcggcctattggttaaaaaatgagctgatttaacaaaaatttaacgcgaattttaacaaaatattaacgtttataatttcaggtggcatctttcggggaaatgtgcgcggaacccctatttgtttatttttctaaatacattcaaatatgtatccgctcatgagacaataaccctgataaatgcttcaataatattgaaaaaggaagagtatgagtattcaacatttccgtgtcgcccttattcccttttttgcggcattttgccttcctgtttttgctcacccagaaacgctggtgaaagtaaaagatgctgaagatcagttgggtgcacgagtgggttacatcgaactggatctcaatagtggtaagatccttgagagttttcgccccgaagaacgttttccaatgatgagcacttttaaagttctgctatgtggcgcggtattatcccgtattgacgccgggcaagagcaactcggtcgccgcatacactattctcagaatgacttggttgagtactcaccagtcacagaaaagcatcttacggatggcatgacagtaagagaattatgcagtgctgccataaccatgagtgataacactgcggccaacttacttctgacaacgatcggaggaccgaaggagctaaccgcttttttgcacaacatgggggatcatgtaactcgccttgatcgttgggaaccggagctgaatgaagccataccaaacgacgagcgtgacaccacgatgcctgtagtaatggtaacaacgttgcgcaaactattaactggcgaactacttactctagcttcccggcaacaattaatagactggatggaggcggataaagttgcaggaccacttctgcgctcggcccttccggctggctggtttattgctgataaatctggagccggtgagcgtgggtctcgcggtatcattgcagcactggggccagatggtaagccctcccgtatcgtagttatctacacgacggggagtcaggcaactatggatgaacgaaatagacagatcgctgagataggtgcctcactgattaagcattggtaactgtcagaccaagtttactcatatatactttagattgatttaaaacttcatttttaatttaaaaggatctaggtgaagatcctttttgataatctcatgaccaaaatcccttaacgtgagttttcgttccactgagcgtcagaccccgtagaaaagatcaaaggatcttcttgagatcctttttttctgcgcgtaatctgctgcttgcaaacaaaaaaaccaccgctaccagcggtggtttgtttgccggatcaagagctaccaactctttttccgaaggtaactggcttcagcagagcgcagataccaaatactgtccttctagtgtagccgtagttaggccaccacttcaagaactctgtagcaccgcctacatacctcgctctgctaatcctgttaccagtggctgctgccagtggcgataagtcgtgtcttaccgggttggactcaagacgatagttaccggataaggcgcagcggtcgggctgaacggggggttcgtgcacacagcccagcttggagcgaacgacctacaccgaactgagatacctacagcgtgagctatgagaaagcgccacgcttcccgaagggagaaaggcggacaggtatccggtaagcggcagggtcggaacaggagagcgcacgagggagcttccagggggaaacgcctggtatctttatagtcctgtcgggtttcgccacctctgacttgagcgtcgatttttgtgatgctcgtcaggggggcggagcctatggaaaaacgccagcaacgcggcctttttacggttcctggccttttgctgcggttttgctcacatgttctttcctgcgttatcccctgattctgtggataaccgtattaccgcctttgagtgagctgataccgctcgccgcagccgaacgaccgagcgcagcgagtcagtgagcgaggaagcggaagagcgcccaatacgcaaaccgcctctccccgcgcgttggccgattcattaatgcagctggcacgacaggtttcccgactggaaagcgggcagtgagcgcaacgcaattaatgtgagttagctcactcattaggcaccccaggctttacactttatgcttccggctcgtatgttgtgtggaattgtgagcggataacaatttcacacaggaaacagctatgaccatgattacgccagatttaattaagg

SEQ ID NO: 6 - DNA, 210 bp, synthetic construct
  misc_feature 1..210: note = KRAB domain
  source 1..210: mol_type = other DNA
  CDS 1..210
gctaagtcactaactgcctggtcccggacactggtgaccttcaaggatgtatttgtggacttcaccagggaggagtggaagctgctggacactgctcagcagatcgtgtacagaaatgtgatgctggagaactataagaacctggtttccttgggttatcagcttactaagccagatgtgatcctccggttggagaagggagaagagccc

SEQ ID NO: 7 - protein, 70 aa, synthetic construct
  REGION 1..70: note = Synthetic Construct
AKSLTAWSRTLVTFKDVFVDFTREEWKLLDTAQQIVYRNVMLENYKNLVSLGYQLTKPDVILRLEKGEEP

SEQ ID NO: 8 - protein, 863 aa, synthetic construct
  REGION 1..863: note = C-Intein-dCCas9
MIKIATRKYLGKQNVYDIGVERDHNFALKNGFIASCFDSVEISGVEDRFNASLGTYHDLLKIIKDKDFLDNEENEDILEDIVLTLTLFEDREMIEERLKTYAHLFDDKVMKQLKRRRYTGWGRLSRKLINGIRDKQSGKTILDFLKSDGFANRNFMQLIHDDSLTFKEDIQKAQVSGQGDSLHEHIANLAGSPAIKKGILQTVKVVDELVKVMGRHKPENIVIEMARENQTTQKGQKNSRERMKRIEEGIKELGSQILKEHPVENTQLQNEKLYLYYLQNGRDMYVDQELDINRLSDYDVDAIVPQSFLKDDSIDNKVLTRSDKNRGKSDNVPSEEVVKKMKNYWRQLLNAKLITQRKFDNLTKAERGGLSELDKAGFIKRQLVETRQITKHVAQILDSRMNTKYDENDKLIREVKVITLKSKLVSDFRKDFQFYKVREINNYHHAHDAYLNAVVGTALIKKYPKLESEFVYGDYKVYDVRKMIAKSEQEIGKATAKYFFYSNIMNFFKTEITLANGEIRKRPLIETNGETGEIVWDKGRDFATVRKVLSMPQVNIVKKTEVQTGGFSKESILPKRNSDKLIARKKDWDPKKYGGFDSPTVAYSVLVVAKVEKGKSKKLKSVKELLGITIMERSSFEKNPIDFLEAKGYKEVKKDLIIKLPKYSLFELENGRKRMLASAGELQKGNELALPSKYVNFLYLASHYEKLKGSPEDNEQKQLFVEQHKHYLDEIIEQISEFSKRVILADANLDKVLSAYNKHRDKPIREQAENIIHLFTLTNLGAPAAFKYFDTTIDRKRYTSTKEVLDATLIHQSITGLYETRIDLSQLGGDAYPYDVPDYASLGSGSPKKKRKVEDPKKKRKVD

SEQ ID NO: 9 - protein, 702 aa, synthetic construct
  REGION 1..702: note = dNCas9-N-Intein
MGPKKKRKVAAADYKDDDDKGIHGVPAADKKYSIGLAIGTNSVGWAVITDEYKVPSKKFKVLGNTDRHSIKKNLIGALLFDSGETAEATRLKRTARRRYTRRKNRICYLQEIFSNEMAKVDDSFFHRLEESFLVEEDKKHERHPIFGNIVDEVAYHEKYPTIYHLRKKLVDSTDKADLRLIYLALAHMIKFRGHFLIEGDLNPDNSDVDKLFIQLVQTYNQLFEENPINASGVDAKAILSARLSKSRRLENLIAQLPGEKKNGLFGNLIALSLGLTPNFKSNFDLAEDAKLQLSKDTYDDDLDNLLAQIGDQYADLFLAAKNLSDAILLSDILRVNTEITKAPLSASMIKRYDEHHQDLTLLKALVRQQLPEKYKEIFFDQSKNGYAGYIDGGASQEEFYKFIKPILEKMDGTEELLVKLNREDLLRKQRTFDNGSIPHQIHLGELHAILRRQEDFYPFLKDNREKIEKILTFRIPYYVGPLARGNSRFAWMTRKSEETITPWNFEEVVDKGASAQSFIERMTNFDKNLPNEKVLPKHSLLYEYFTVYNELTKVKYVTEGMRKPAFLSGEQKKAIVDLLFKTNRKVTVKQLKEDYFKKIECLSYETEILTVEYGLLPIGKIVEKRIECTVYSVDNNGNIYTQPVAQWHDRGEQEVFEYCLEDGSLIRATKDHKFMTVDGQMLPIDEIFERELDLMRVDNLPN

SEQ ID NO: 10 - DNA, 7501 bp, synthetic construct
  misc_feature 1..7501: note = AAV,dNCas9-KRAB
  source 1..7501: mol_type = other DNA
ctgcgcgctcgctcgctcactgaggccgcccgggcaaagcccgggcgtcgggcgacctttggtcgcccggcctcagtgagcgagcgagcgcgcagagagggagtggccaactccatcactaggggttccttgtagttaatgattaacccgccatgctacttatctacgtagccatgctctaggaagatcggaattcgcccttaagctagctagttattaatagtaatcaattacggggtcattagttcatagcccatatatggagttccgcgttacataacttacggtaaatggcccgcctggctgaccgcccaacgacccccgcccattgacgtcaataatgacgtatgttcccatagtaacgccaatagggactttccattgacgtcaatgggtggagtatttacggtaaactgcccacttggcagtacatcaagtgtatcatatgccaagtacgccccctattgacgtcaatgacggtaaatggcccgcctggcattatgcccagtacatgaccttatgggactttcctacttggcagtacatctacgtattagtcatcgctattaccatggtgatgcggttttggcagtacatcaatgggcgtggatagcggtttgactcacggggatttccaagtctccaccccattgacgtcaatgggagtttgttttggcaccaaaatcaacgggactttccaaaatgtcgtaacaactccgccccattgacgcaaatgggcggtaggcgtgtacggtgggaggtctatataagcagagctggtttagtgaaccgtcagatcctgcagaagttggtcgtgaggcactgggcaggtaagtatcaaggttacaagacaggtttaaggagaccaatagaaactgggcttgtcgagacagagaagactcttgcgtttctgataggcacctattggtcttactgacatccactttgcctttctctccacaggtgtccaggcggccgcatggatatcgccaccatggatgctaagtcactaactgcctggtcccggacactggtgaccttcaaggatgtatttgtggacttcaccagggaggagtggaagctgctggacactgctcagcagatcgtgtacagaaatgtgatgctggagaactataagaacctggtttccttgggttatcagcttactaagccagatgtgatcctccggttggagaagggagaagagcccggcggttccggcggagggtcggatatcatgggccccaagaaaaaacgcaaggtggccgcagcagactataaggatgacgacgataaggggatccatggtgtgcctgctgcagataaaaaatacagcatcggcctggctatcggaactaactccgtcggctgggccgtcattaccgacgaatacaaagtacctagcaaaaagttcaaggtgcttggcaacacagatcgccactcaatcaagaaaaaccttatcggagccctgctgtttgactcaggcgaaaccgccgaggctacacgcctgaaaagaacagctagacggcggtacaccagaaggaagaaccggatctgttatcttcaggagattttctccaatgagatggctaaggtggacgattctttcttccatcgactcgaagaatctttcttggtggaggaagataagaaacacgagaggcatcctattttcggaaacattgtcgatgaagtggcctatcatgagaaataccccacgatctaccatctgcgaaaaaagttggttgactctaccgacaaggcggacctgaggcttatttatctggccctggcccatatgatcaaattcagggggcacttcttgatcgagggggaccttaatcccgacaactctgacgtggataagttgttcatacagcttgtgcagacctacaaccagctgttcgaggagaatccaatcaacgccagcggagtggacgctaaagccattctgagcgcgagattgagcaagtctagaagattggaaaaccttatagcccagctgccaggtgagaagaagaacggactgtttggcaatctcattgcgcttagcctcggactcaccccgaacttcaaatccaacttcgacctcgccgaagatgccaaattgcagctcagtaaggatacgtatgacgatgatcttgacaatctgctggcgcagatcggggaccagtacgccgatcttttcttggcagcaaaaaatctctcagatgcaatactcttgtcagacatactgcgagttaataccgagattactaaggctccgctttctgcctccatgatcaagcgctacgatgagcatcaccaggatctgacactgttgaaagccctggtgcgccaacagctgccagagaaatacaaggaaatcttttttgaccagtccaagaatggctacgcaggatacatcgatggaggagccagtcaggaggaattttacaagtttattaagcctatcctggagaagatggatggtaccgaagaactcctggtcaagctcaaccgagaagatttgcttcgcaagcaaaggacttttgacaacggctccattccgcatcagattcatctgggcgagctgcatgccattctgcgaagacaggaggatttttacccatttctgaaggacaaccgagagaagatcgagaaaatactgacattcaggataccatattacgtgggtccactcgccaggggcaactcccgattcgcctggatgacaaggaaaagcgaagagacgatcactccatggaacttcgaggaggtcgtggacaagggggcctccgcgcagagctttatcgagaggatgacgaactttgacaaaaatctccctaacgagaaggtgctgccaaaacattctctgctctacgagtatttcaccgtttataatgagctcacaaaggtgaagtacgtgaccgaagggatgcggaagcccgcttttctgtccggagagcagaagaaggctatcgtggatttgctctttaagactaaccgcaaggtaacagtcaagcagctgaaggaagactacttcaagaagatcgaatgcttgtcctacgaaacggaaatcttgacagttgagtacgggctcctgccaatcgggaagatagtagagaagaggattgaatgtaccgtctattctgttgataacaacggtaacatatacacccagcccgtcgcccaatggcacgatcgcggtgagcaggaggtgttcgaatactgtctggaggacgggtcattgattcgggcgactaaggaccataagtttatgacggtagacggccagatgttgcccatagatgagatctttgagcgggaactcgacttgatgagagtcgataatcttcctaattaaaccggagcttggatccaatcaacctctggattacaaaatttgtgaaagattgactggtattcttaactatgttgctccttttacgctatgtggatacgctgctttaatgcctttgtatcatgctattgcttcccgtatggctttcattttctcctccttgtataaatcctggttgctgtctctttatgaggagttgtggcccgttgtcaggcaacgtggcgtggtgtgcactgtgtttgctgacgcaacccccactggttggggcattgccaccacctgtcagctcctttccgggactttcgctttccccctccctattgccacggcggaactcatcgccgcctgccttgcccgctgctggacaggggctcggctgttgggcactgacaattccgtggtgttgtcggggaaatcatcgtcctttccttggctgctcgcctgtgttgccacctggattctgcgcgggacgtccttctgctacgtcccttcggccctcaatccagcggaccttccttcccgcggcctgctgccggctctgcggcctcttccgcgtcttcgagatctgcctcgactgtgccttctagttgccagccatctgttgtttgcccctcccccgtgccttccttgaccctggaaggtgccactcccactgtcctttcctaataaaatgaggaaattgcatcgcattgtctgagtaggtgtcattctattctggggggtggggtggggcaggacagcaagggggaggattgggaagacaatagcaggcatgctggggactcgagacgcgtggaggagggcctatttcccatgattccttcatatttgcatatacgatacaaggctgttagagagataattagaattaatttgactgtaaacacaaagatattagtacaaaatacgtgacgtagaaagtaataatttcttgggtagtttgcagttttaaaattatgttttaaaatggactatcatatgcttaccgtaacttgaaagtatttcgatttcttggctttatatatcttgtggaaaggacgaaacaccggttttagagctagaaatagcaagttaaaataaggctagtccgttatcaacttgaaaaagtggcaccgagtcggtgcttttttctcgagttaagggcgaattcccgataaggatcttcctagagcatggctacgtagataagtagcatggcgggttaatcattaactacaaggaacccctagtgatggagttggccactccctctctgcgcgctcgctcgctcactgaggccgggcgaccaaaggtcgcccgacgcccgggctttgcccgggcggcctcagtgagcgagcgagcgcgcagccttaattaacctaattcactggccgtcgttttacaacgtcgtgactgggaaaaccctggcgttacccaacttaatcgccttgcagcacatccccctttcgccagctggcgtaatagcgaagaggcccgcaccgatcgcccttcccaacagttgcgcagcctgaatggcgaatgggacgcgccctgtagcggcgcattaagcgcggcgggtgtggtggttacgcgcagcgtgaccgctacacttgccagcgccctagcgcccgctcctttcgctttcttcccttcctttctcgccacgttcgccggctttccccgtcaagctctaaatcgggggctccctttagggttccgatttagtgctttacggcacctcgaccccaaaaaacttgattagggtgatggttcacgtagtgggccatcgccctgatagacggtttttcgccctttgacgttggagtccacgttctttaatagtggactcttgttccaaactggaacaacactcaaccctatctcggtctattcttttgatttataagggattttgccgatttcggcctattggttaaaaaatgagctgatttaacaaaaatttaacgcgaattttaacaaaatattaacgtttataatttcaggtggcatctttcggggaaatgtgcgcggaacccctatttgtttatttttctaaatacattcaaatatgtatccgctcatgagacaataaccctgataaatgcttcaataatattgaaaaaggaagagtatgagtattcaacatttccgtgtcgcccttattcccttttttgcggcattttgccttcctgtttttgctcacccagaaacgctggtgaaagtaaaagatgctgaagatcagttgggtgcacgagtgggttacatcgaactggatctcaatagtggtaagatccttgagagttttcgccccgaagaacgttttccaatgatgagcacttttaaagttctgctatgtggcgcggtattatcccgtattgacgccgggcaagagcaactcggtcgccgcatacactattctcagaatgacttggttgagtactcaccagtcacagaaaagcatcttacggatggcatgacagtaagagaattatgcagtgctgccataaccatgagtgataacactgcggccaacttacttctgacaacgatcggaggaccgaaggagctaaccgcttttttgcacaacatgggggatcatgtaactcgccttgatcgttgggaaccggagctgaatgaagccataccaaacgacgagcgtgacaccacgatgcctgtagtaatggtaacaacgttgcgcaaactattaactggcgaactacttactctagcttcccggcaacaattaatagactggatggaggcggataaagttgcaggaccacttctgcgctcggcccttccggctggctggtttattgctgataaatctggagccggtgagcgtgggtctcgcggtatcattgcagcactggggccagatggtaagccctcccgtatcgtagttatctacacgacggggagtcaggcaactatggatgaacgaaatagacagatcgctgagataggtgcctcactgattaagcattggtaactgtcagaccaagtttactcatatatactttagattgatttaaaacttcatttttaatttaaaaggatctaggtgaagatcctttttgataatctcatgaccaaaatcccttaacgtgagttttcgttccactgagcgtcagaccccgtagaaaagatcaaaggatcttcttgagatcctttttttctgcgcgtaatctgctgcttgcaaacaaaaaaaccaccgctaccagcggtggtttgtttgccggatcaagagctaccaactctttttccgaaggtaactggcttcagcagagcgcagataccaaatactgtccttctagtgtagccgtagttaggccaccacttcaagaactctgtagcaccgcctacatacctcgctctgctaatcctgttaccagtggctgctgccagtggcgataagtcgtgtcttaccgggttggactcaagacgatagttaccggataaggcgcagcggtcgggctgaacggggggttcgtgcacacagcccagcttggagcgaacgacctacaccgaactgagatacctacagcgtgagctatgagaaagcgccacgcttcccgaagggagaaaggcggacaggtatccggtaagcggcagggtcggaacaggagagcgcacgagggagcttccagggggaaacgcctggtatctttatagtcctgtcgggtttcgccacctctgacttgagcgtcgatttttgtgatgctcgtcaggggggcggagcctatggaaaaacgccagcaacgcggcctttttacggttcctggccttttgctgcggttttgctcacatgttctttcctgcgttatcccctgattctgtggataaccgtattaccgcctttgagtgagctgataccgctcgccgcagccgaacgaccgagcgcagcgagtcagtgagcgaggaagcggaagagcgcccaatacgcaaaccgcctctccccgcgcgttggccgattcattaatgcagctggcacgacaggtttcccgactggaaagcgggcagtgagcgcaacgcaattaatgtgagttagctcactcattaggcaccccaggctttacactttatgcttccggctcgtatgttgtgtggaattgtgagcggataacaatttcacacaggaaacagctatgaccatgattacgccagatttaattaagg

SEQ ID NO: 11 - DNA, 19 bp, synthetic construct
  misc_feature 1..19: note = gRNA spacer sequence
  source 1..19: mol_type = other DNA
acagtgggcaggattgaaa

SEQ ID NO: 12 - DNA, 19 bp, synthetic construct
  misc_feature 1..19: note = gRNA spacer sequence
  source 1..19: mol_type = other DNA
gcaggtgcactcaccgggt

SEQ ID NO: 13 - DNA, 20 bp, synthetic construct
  misc_feature 1..20: note = gRNA spacer sequence
  source 1..20: mol_type = other DNA
gagctcagggagcatcgagg

SEQ ID NO: 14 - DNA, 19 bp, synthetic construct
  misc_feature 1..19: note = gRNA spacer sequence
  source 1..19: mol_type = other DNA
agagtcgcaattggagcgc

SEQ ID NO: 15 - DNA, 19 bp, synthetic construct
  misc_feature 1..19: note = gRNA spacer sequence
  source 1..19: mol_type = other DNA
ccagaccagcctgcacagt

SEQ ID NO: 16 - DNA, 20 bp, synthetic construct
  misc_feature 1..20: note = gRNA spacer sequence
  source 1..20: mol_type = other DNA
gagcgcaggctaggcctgca

SEQ ID NO: 17 - DNA, 19 bp, synthetic construct
  misc_feature 1..19: note = gRNA spacer sequence
  source 1..19: mol_type = other DNA
ctaggagtccgggataccc

SEQ ID NO: 18 - DNA, 20 bp, synthetic construct
  misc_feature 1..20: note = gRNA spacer sequence
  source 1..20: mol_type = other DNA
gaatccgcaggtgcactcac

SEQ ID NO: 19 - DNA, 20 bp, synthetic construct
  misc_feature 1..20: note = gRNA spacer sequence
  source 1..20: mol_type = other DNA
gaccagcctgcacagtgggc

SEQ ID NO: 20 - DNA, 20 bp, synthetic construct
  misc_feature 1..20: note = gRNA spacer sequence
  source 1..20: mol_type = other DNA
gcgacgcggttggcagccga

SEQ ID NO: 21 - DNA, 20 bp, synthetic construct
  misc_feature 1..20: note = gRNA spacer sequence
  source 1..20: mol_type = other DNA
ggtcgccagcgctccagcgg

SEQ ID NO: 22 - DNA, 20 bp, synthetic construct
  misc_feature 1..20: note = gRNA spacer sequence
  source 1..20: mol_type = other DNA
gctttccaattccgccagct

SEQ ID NO: 23 - DNA, 20 bp, synthetic construct
  misc_feature 1..20: note = gRNA spacer sequence
  source 1..20: mol_type = other DNA
caattccgccagctcggctg

SEQ ID NO: 24 - DNA, 20 bp, synthetic construct
  misc_feature 1..20: note = gRNA spacer sequence
  source 1..20: mol_type = other DNA
cccagcctcagccgagctgg

SEQ ID NO: 25 - DNA, 20 bp, synthetic construct
  misc_feature 1..20: note = gRNA spacer sequence
  source 1..20: mol_type = other DNA
ccgccagctcggctgaggct

SEQ ID NO: 26 - DNA, 20 bp, synthetic construct
  misc_feature 1..20: note = gRNA spacer sequence
  source 1..20: mol_type = other DNA
ggaaagccgacagccgccgc

SEQ ID NO: 27 - DNA, 20 bp, synthetic construct
  misc_feature 1..20: note = gRNA spacer sequence
  source 1..20: mol_type = other DNA
agcgctccagcggcggctgt

SEQ ID NO: 28 - DNA, 20 bp, synthetic construct
  misc_feature 1..20: note = gRNA spacer sequence
  source 1..20: mol_type = other DNA
ggcggtcgccagcgctccag

SEQ ID NO: 29 - DNA, 20 bp, synthetic construct
  misc_feature 1..20: note = gRNA spacer sequence
  source 1..20: mol_type = other DNA
ctcagccgagctggcggaat

SEQ ID NO: 30 - DNA, 20 bp, synthetic construct
  misc_feature 1..20: note = gRNA spacer sequence
  source 1..20: mol_type = other DNA
tagcccagcctcagccgagc

SEQ ID NO: 31 - DNA, 20 bp, synthetic construct
  misc_feature 1..20: note = gRNA spacer sequence
  source 1..20: mol_type = other DNA
ggcggtcgccagcgctccag

SEQ ID NO: 32 - DNA, 20 bp, synthetic construct
  misc_feature 1..20: note = gRNA spacer sequence
  source 1..20: mol_type = other DNA
gccacctggaaagaagagag

SEQ ID NO: 33 - DNA, 20 bp, synthetic construct
  misc_feature 1..20: note = gRNA spacer sequence
  source 1..20: mol_type = other DNA
ggtcgccagcgctccagcgg

SEQ ID NO: 34 - DNA, 20 bp, synthetic construct
  misc_feature 1..20: note = gRNA spacer sequence
  source 1..20: mol_type = other DNA
gccagcaatgggaggaagaa

SEQ ID NO: 35 - DNA, 20 bp, synthetic construct
  misc_feature 1..20: note = gRNA spacer sequence
  source 1..20: mol_type = other DNA
gttccaggtggcgtaataca

SEQ ID NO: 36 - DNA, 20 bp, synthetic construct
  misc_feature 1..20: note = gRNA spacer sequence
  source 1..20: mol_type = other DNA
ggcggggctgctacctccac

SEQ ID NO: 37 - DNA, 20 bp, synthetic construct
  misc_feature 1..20: note = gRNA spacer sequence
  source 1..20: mol_type = other DNA
gggcgcagtctgcttgcagg

SEQ ID NO: 38 - DNA, 20 bp, synthetic construct
  misc_feature 1..20: note = gRNA spacer sequence
  source 1..20: mol_type = other DNA
ggcgctccagcggcggctgt

SEQ ID NO: 39 - DNA, 20 bp, synthetic construct
  misc_feature 1..20: note = gRNA spacer sequence
  source 1..20: mol_type = other DNA
gaccgggtggttccagcaat

SEQ ID NO: 40 - DNA, 20 bp, synthetic construct
  misc_feature 1..20: note = gRNA spacer sequence
  source 1..20: mol_type = other DNA
ggggtggttccagcaatggg

SEQ ID NO: 41 - DNA, 20 bp, synthetic construct
  misc_feature 1..20: note = gRNA spacer sequence
  source 1..20: mol_type = other DNA
gggcgcagtctgcttgcagg

SEQ ID NO: 42 - DNA, 20 bp, synthetic construct
  misc_feature 1..20: note = gRNA spacer sequence
  source 1..20: mol_type = other DNA
tgggtgccagtggctgctag

SEQ ID NO: 43 - DNA, 20 bp, synthetic construct
  misc_feature 1..20: note = gRNA spacer sequence
  source 1..20: mol_type = other DNA
tctgggctcctgttgctcag

SEQ ID NO: 44 - DNA, 20 bp, synthetic construct
  misc_feature 1..20: note = gRNA spacer sequence
  source 1..20: mol_type = other DNA
gcagccctgagagagcgccg

SEQ ID NO: 45 - DNA, 20 bp, synthetic construct
  misc_feature 1..20: note = gRNA spacer sequence
  source 1..20: mol_type = other DNA
gagcacgggcgaaagaccga

SEQ ID NO: 46 - DNA, 20 bp, synthetic construct
  misc_feature 1..20: note = gRNA spacer sequence
  source 1..20: mol_type = other DNA
atagacacaggtgggtgtgg

SEQ ID NO: 47 - DNA, 20 bp, synthetic construct
  misc_feature 1..20: note = gRNA spacer sequence
  source 1..20: mol_type = other DNA
atgtgaaaatagacacaggt

SEQ ID NO: 48 - DNA, 20 bp, synthetic construct
  misc_feature 1..20: note = gRNA spacer sequence
  source 1..20: mol_type = other DNA
gatgtgaaaatagacacagg

SEQ ID NO: 49 - DNA, 20 bp, synthetic construct
  misc_feature 1..20: note = gRNA spacer sequence
  source 1..20: mol_type = other DNA
cgagatgtgaaaatagacac

SEQ ID NO: 50 - DNA, 20 bp, synthetic construct
  misc_feature 1..20: note = gRNA spacer sequence
  source 1..20: mol_type = other DNA
gccacctggaaagaagagag

SEQ ID NO: 51 - DNA, 20 bp, synthetic construct
  misc_feature 1..20: note = gRNA spacer sequence
  source 1..20: mol_type = other DNA
aggggagaagcttgaccggg

SEQ ID NO: 52 - DNA, 20 bp, synthetic construct
  misc_feature 1..20: note = gRNA spacer sequence
  source 1..20: mol_type = other DNA
cgggtggttccagcaatggg

SEQ ID NO: 53 - DNA, 20 bp, synthetic construct
  misc_feature 1..20: note = gRNA spacer sequence
  source 1..20: mol_type = other DNA
atagctgggcagctcctgtg

SEQ ID NO: 54 - DNA, 20 bp, synthetic construct
  misc_feature 1..20: note = gRNA spacer sequence
  source 1..20: mol_type = other DNA
ccacagagtcaaaaccgcac

SEQ ID NO: 55 - DNA, 20 bp, synthetic construct
  misc_feature 1..20: note = gRNA spacer sequence
  source 1..20: mol_type = other DNA
gctgccaggttctgaaactg

SEQ ID NO: 56 - DNA, 20 bp, synthetic construct
  misc_feature 1..20: note = gRNA spacer sequence
  source 1..20: mol_type = other DNA
caggttctgaaactgtggaa

SEQ ID NO: 57 - DNA, 20 bp, synthetic construct
  misc_feature 1..20: note = gRNA spacer sequence
  source 1..20: mol_type = other DNA
aaaggaagggtagcaatgcc

SEQ ID NO: 58 - DNA, 20 bp, synthetic construct
  misc_feature 1..20: note = gRNA spacer sequence
  source 1..20: mol_type = other DNA
ggaagggtagcaatgcctgg

SEQ ID NO: 59 - DNA, 20 bp, synthetic construct
  misc_feature 1..20: note = gRNA spacer sequence
  source 1..20: mol_type = other DNA
ataaaagacagtaaaccacc

SEQ ID NO: 60 - DNA, 20 bp, synthetic construct
  misc_feature 1..20: note = gRNA spacer sequence
  source 1..20: mol_type = other DNA
tagatggacttcaattcaag

SEQ ID NO: 61 - DNA, 20 bp, synthetic construct
  misc_feature 1..20: note = gRNA spacer sequence
  source 1..20: mol_type = other DNA
gcttagcagatacaacctgt

SEQ ID NO: 62 - DNA, 20 bp, synthetic construct
  misc_feature 1..20: note = gRNA spacer sequence
  source 1..20: mol_type = other DNA
cttagcagatacaacctgtg

SEQ ID NO: 63 - DNA, 20 bp, synthetic construct
  misc_feature 1..20: note = gRNA spacer sequence
  source 1..20: mol_type = other DNA
aatttacatgagaaacttag

SEQ ID NO: 64 - DNA, 20 bp, synthetic construct
  misc_feature 1..20: note = gRNA spacer sequence
  source 1..20: mol_type = other DNA
atttacatgagaaacttagg

SEQ ID NO: 65 - DNA, 20 bp, synthetic construct
  misc_feature 1..20: note = gRNA spacer sequence
  source 1..20: mol_type = other DNA
tttacatgagaaacttaggg

SEQ ID NO: 66 - DNA, 20 bp, synthetic construct
  misc_feature 1..20: note = gRNA spacer sequence
  source 1..20: mol_type = other DNA
tcatgaaaatttgcgacaca

SEQ ID NO: 67 - DNA, 20 bp, synthetic construct
  misc_feature 1..20: note = gRNA spacer sequence
  source 1..20: mol_type = other DNA
tgattatatgcaggccctag

SEQ ID NO: 68 - DNA, 20 bp, synthetic construct
  misc_feature 1..20: note = gRNA spacer sequence
  source 1..20: mol_type = other DNA
taatcatgggagcccttctg

SEQ ID NO: 69 - DNA, 20 bp, synthetic construct
  misc_feature 1..20: note = gRNA spacer sequence
  source 1..20: mol_type = other DNA
atagaagcattaccacagaa

SEQ ID NO: 70 - DNA, 20 bp, synthetic construct
  misc_feature 1..20: note = gRNA spacer sequence
  source 1..20: mol_type = other DNA
taatcaacccactttctctg

SEQ ID NO: 71 - DNA, 20 bp, synthetic construct
  misc_feature 1..20: note = gRNA spacer sequence
  source 1..20: mol_type = other DNA
aacccactttctctgtggca

SEQ ID NO: 72 - DNA, 20 bp, synthetic construct
  misc_feature 1..20: note = gRNA spacer sequence
  source 1..20: mol_type = other DNA
gccgtgtagatacagaaaag

SEQ ID NO: 73 - DNA, 20 bp, synthetic construct
  misc_feature 1..20: note = gRNA spacer sequence
  source 1..20: mol_type = other DNA
gtatagagaatgaattgcag

SEQ ID NO: 74 - DNA, 20 bp, synthetic construct
  misc_feature 1..20: note = gRNA spacer sequence
  source 1..20: mol_type = other DNA
tgtatagagaatgaattgca

SEQ ID NO: 75 - DNA, 20 bp, synthetic construct
  misc_feature 1..20: note = gRNA spacer sequence
  source 1..20: mol_type = other DNA
atttaaaaaaaaaaaaaaag

SEQ ID NO: 76 - DNA, 20 bp, synthetic construct
  misc_feature 1..20: note = gRNA spacer sequence
  source 1..20: mol_type = other DNA
agagagtaaaccatatgctg

SEQ ID NO: 77 - DNA, 20 bp, synthetic construct
  misc_feature 1..20: note = gRNA spacer sequence
  source 1..20: mol_type = other DNA
gaagagaataggttctggtg

SEQ ID NO: 78 - DNA, 20 bp, synthetic construct
  misc_feature 1..20: note = gRNA spacer sequence
  source 1..20: mol_type = other DNA
atgtgttttagccacgacct

SEQ ID NO: 79 - DNA, 20 bp, synthetic construct
  misc_feature 1..20: note = gRNA spacer sequence
  source 1..20: mol_type = other DNA
tccaacatcaagaccaacac

SEQ ID NO: 80 - DNA, 20 bp, synthetic construct
  misc_feature 1..20: note = gRNA spacer sequence
  source 1..20: mol_type = other DNA
ttccaacatcaagaccaaca

SEQ ID NO: 81 - DNA, 20 bp, synthetic construct
  misc_feature 1..20: note = gRNA spacer sequence
  source 1..20: mol_type = other DNA
tttgcataccaaatactcca

SEQ ID NO: 82 - DNA, 20 bp, Artificial Sequence
  misc_feature 1..20: note = gRNA spacer sequence
  source 1..20: mol_type = other DNA
ttgcataccaaatactccaa

SEQ ID NO: 83 - DNA, 20 bp, synthetic construct
  misc_feature 1..20: note = gRNA spacer sequence
  source 1..20: mol_type = other DNA
gcctggcatcaagtagtagg

SEQ ID NO: 84 - DNA, 20 bp, synthetic construct
  misc_feature 1..20: note = gRNA spacer sequence
  source 1..20: mol_type = other DNA
atcatggtatgatattgagg

SEQ ID NO: 85 - DNA, 20 bp, synthetic construct
  misc_feature 1..20: note = gRNA spacer sequence
  source 1..20: mol_type = other DNA
agaaatgtagtcagatgagg

SEQ ID NO: 86 - DNA, 20 bp, synthetic construct
  misc_feature 1..20: note = gRNA spacer sequence
  source 1..20: mol_type = other DNA
ccataagttaggtttccaca

SEQ ID NO: 87 - DNA, 20 bp, synthetic construct
  misc_feature 1..20: note = gRNA spacer sequence
  source 1..20: mol_type = other DNA
aaacatcaatttagaccgtg

SEQ ID NO: 88 - DNA, 20 bp, synthetic construct
  misc_feature 1..20: note = gRNA spacer sequence
  source 1..20: mol_type = other DNA
tctctaaggaaggttcagag

SEQ ID NO: 89 - DNA, 20 bp, synthetic construct
  misc_feature 1..20: note = gRNA spacer sequence
  source 1..20: mol_type = other DNA
gaaggttcagagaggcaatg

SEQ ID NO: 90 - DNA, 20 bp, synthetic construct
  misc_feature 1..20: note = gRNA spacer sequence
  source 1..20: mol_type = other DNA
atagtctgcaaaaataaagg

SEQ ID NO: 91 - DNA, 20 bp, synthetic construct
  misc_feature 1..20: note = gRNA spacer sequence
  source 1..20: mol_type = other DNA
aattatttaccaaaaatctg

SEQ ID NO: 92 - DNA, 20 bp, synthetic construct
  misc_feature 1..20: note = gRNA spacer sequence
  source 1..20: mol_type = other DNA
attgtggatgttgtattgga

SEQ ID NO: 93 - DNA, 20 bp, synthetic construct
  misc_feature 1..20: note = gRNA spacer sequence
  source 1..20: mol_type = other DNA
aggaatgaaacccttctggg

SEQ ID NO: 94 - DNA, 20 bp, synthetic construct
  misc_feature 1..20: note = gRNA spacer sequence
  source 1..20: mol_type = other DNA
tgccaggccatgataaagtg

SEQ ID NO: 95 - DNA, 20 bp, synthetic construct
  misc_feature 1..20: note = gRNA spacer sequence
  source 1..20: mol_type = other DNA
acaggagcccagagaaaaag

SEQ ID NO: 96 - DNA, 20 bp, synthetic construct
  misc_feature 1..20: note = gRNA spacer sequence
  source 1..20: mol_type = other DNA
ggagcccagagaaaaagaag

SEQ ID NO: 97 - DNA, 20 bp, synthetic construct
  misc_feature 1..20: note = gRNA spacer sequence
  source 1..20: mol_type = other DNA
acagagtcaaaaccgcacag

SEQ ID NO: 98 - DNA, 20 bp, synthetic construct
  misc_feature 1..20: note = gRNA spacer sequence
  source 1..20: mol_type = other DNA
gcgtaaacagaaataaaaga

SEQ ID NO: 99 - DNA, 20 bp, synthetic construct
  misc_feature 1..20: note = gRNA spacer sequence
  source 1..20: mol_type = other DNA
tctgcgctgagaaatagggg

SEQ ID NO: 100 - DNA, 20 bp, synthetic construct
  misc_feature 1..20: note = gRNA spacer sequence
  source 1..20: mol_type = other DNA
tttgcttctgaaactcagca

SEQ ID NO: 101 - DNA, 20 bp, synthetic construct
  misc_feature 1..20: note = gRNA spacer sequence
  source 1..20: mol_type = other DNA
gttgctgtgctgagtttcag

SEQ ID NO: 102 - DNA, 20 bp, synthetic construct
  misc_feature 1..20: note = gRNA spacer sequence
  source 1..20: mol_type = other DNA
ctacttttttccttgccaca

SEQ ID NO: 103 - DNA, 20 bp, synthetic construct
  misc_feature 1..20: note = gRNA spacer sequence
  source 1..20: mol_type = other DNA
gctgaaatggagtaataagg

SEQ ID NO: 104 - DNA, 20 bp, synthetic construct
  misc_feature 1..20: note = gRNA spacer sequence
  source 1..20: mol_type = other DNA
atagagaatgaattgcaggg

SEQ ID NO: 105 - DNA, 20 bp, synthetic construct
  misc_feature 1..20: note = gRNA spacer sequence
  source 1..20: mol_type = other DNA
gaatagtgcctggcatcaag

SEQ ID NO: 106 - DNA, 20 bp, synthetic construct
  misc_feature 1..20: note = gRNA spacer sequence
  source 1..20: mol_type = other DNA
gtaatgcattcttagaaagg

SEQ ID NO: 107 - DNA, 20 bp, synthetic construct
  misc_feature 1..20: note = gRNA spacer sequence
  source 1..20: mol_type = other DNA
gtagagttagattaccactt

SEQ ID NO: 108 - DNA, 28 bp, synthetic construct
  misc_feature 1..28: note = murine ZF target sequence
  source 1..28: mol_type = other DNA
tgagtgacggacgggtgaggtttccgtc

SEQ ID NO: 109 - DNA, 28 bp, synthetic construct
  misc_feature 1..28: note = murine ZF target sequence
  misc_feature 25..28: note = n is a, c, g, or t
  source 1..28: mol_type = other DNA
ttcgtggaggagccccggacaagtnnnn

SEQ ID NO: 110 - DNA, 28 bp, synthetic construct
  misc_feature 1..28: note = murine ZF target sequence
  source 1..28: mol_type = other DNA
atggtgctccagaaagtacactctgaat

SEQ ID NO: 111 - DNA, 28 bp, synthetic construct
  misc_feature 1..28: note = murine ZF target sequence
  source 1..28: mol_type = other DNA
tgagtgacggacgggtgaggtttccgtc

SEQ ID NO: 112 - DNA, 18 bp, synthetic construct
  misc_feature 1..18: note = human ZF target sequence
  source 1..18: mol_type = other DNA
agtctgcttgcaggcggt

SEQ ID NO: 113 - DNA, 18 bp, synthetic construct
  misc_feature 1..18: note = human ZF target sequence
  source 1..18: mol_type = other DNA
ccagcggcggctgtcggc

SEQ ID NO: 114 - DNA, 18 bp, synthetic construct
  misc_feature 1..18: note = human ZF target sequence
  source 1..18: mol_type = other DNA
gcctgggtgccagtggct

SEQ ID NO: 115 - DNA, 18 bp, synthetic construct
  misc_feature 1..18: note = human ZF target sequence
  source 1..18: mol_type = other DNA
tggctgctagcggcaggc

SEQ ID NO: 116 - DNA, 18 bp, synthetic construct
  misc_feature 1..18: note = human ZF target sequence
  source 1..18: mol_type = other DNA
gcgtcccctgagcaacag

SEQ ID NO: 117 - DNA, 18 bp, synthetic construct
  misc_feature 1..18: note = human ZF target sequence
  source 1..18: mol_type = other DNA
aaggagaggcccgcgccc

SEQ ID NO: 118 - DNA, 18 bp, synthetic construct
  misc_feature 1..18: note = human ZF target sequence
  source 1..18: mol_type = other DNA
gcaggtgcactgggtggg

SEQ ID NO: 119 - DNA, 18 bp, synthetic construct
  misc_feature 1..18: note = human ZF target sequence
  source 1..18: mol_type = other DNA
gcgcccgtggaggtagca

SEQ ID NO: 120 - DNA, 18 bp, synthetic construct
  misc_feature 1..18: note = human ZF target sequence
  source 1..18: mol_type = other DNA
tgccagggcgcgcccgtg

SEQ ID NO: 121 - DNA, 18 bp, synthetic construct
  misc_feature 1..18: note = human ZF target sequence
  source 1..18: mol_type = other DNA
acagccgccgctggagcg

SEQ ID NO: 122 - DNA, 18 bp, synthetic construct
  misc_feature 1..18: note = human ZF target sequence
  source 1..18: mol_type = other DNA
ccaggagagggcgcgggc

SEQ ID NO: 123 - protein, 295 aa, synthetic construct
  REGION 1..295: note = ZF-KRAB sequence
MDYKDHDGDYKDHDIDYKDDDDKMAPKKKRKVGIHGVPAAMAERPFQCRICMRNFSRSDHLSQHIRTHTGEKPFACDICGRKFARSAVRKNHTKIHTGSQKPFQCRICMRNFSRSDHLSEHIRTHTGEKPFACDICGRKFAQSHHRKTHTKIHTGSQKPFQCRICMRNFSDRSNLSRHIRTHTGEKPFACDICGRKFALKQHLNEHTKIHLRQKDAARGSRTLVTFKDVFVDFTREEWKLLDTAQQIVYRNVMLENYKNLVSLGYQLTKPDVILRLEKGEEPWLVDYKDDDDKRS

SEQ ID NO: 124 - protein, 295 aa, synthetic construct
  REGION 1..295: note = ZF-KRAB sequence
MDYKDHDGDYKDHDIDYKDDDDKMAPKKKRKVGIHGVPAAMAERPFQCRICMRNFSDRSNLSRHIRTHTGEKPFACDICGRKFARSDDRKTHTKIHTGSQKPFQCRICMRNFSERGTLARHIRTHTGEKPFACDICGRKFAQSGHLSRHTKIHTGSQKPFQCRICMRNFSQSGHLARHIRTHTGEKPFACDICGRKFAVSHHLRDHTKIHLRQKDAARGSRTLVTFKDVFVDFTREEWKLLDTAQQIVYRNVMLENYKNLVSLGYQLTKPDVILRLEKGEEPWLVDYKDDDDKRS

SEQ ID NO: 125 - protein, 295 aa, synthetic construct
  REGION 1..295: note = ZF-KRAB sequence
MDYKDHDGDYKDHDIDYKDDDDKMAPKKKRKVGIHGVPAAMAERPFQCRICMRNFSQSGDLTRHIRTHTGEKPFACDICGRKFALAHHLVQHTKIHTGSQKPFQCRICMRNFSQSGNLARHIRTHTGEKPFACDICGRKFAQRIDLTRHTKIHTGSQKPFQCRICMRNFSQSSDLSRHIRTHTGEKPFACDICGRKFAWHSSLHQHTKIHLRQKDAARGSRTLVTFKDVFVDFTREEWKLLDTAQQIVYRNVMLENYKNLVSLGYQLTKPDVILRLEKGEEPWLVDYKDDDDKRS

SEQ ID NO: 126 - protein, 295 aa, synthetic construct
  REGION 1..295: note = ZF-KRAB sequence
MDYKDHDGDYKDHDIDYKDDDDKMAPKKKRKVGIHGVPAAMAERPFQCRICMRNFSQSGNHIRTHTGEKPFACDICGRKFATRNGLKYHTKIHTGSQKPFQCRICMRNFSQSSDLSRHIRLARHIRTHTGEKPFACDICGRKFARLDILQQHTKIHTGSQKPFQCRICMRNFSRSDVLSETHTGEKPFACDICGRKFARKYYLAKHTKIHLRQKDAARGSRTLVTFKDVFVDFTREEWKLLDTAQQIVYRNVMLENYKNLVSLGYQLTKPDVILRLEKGEEPWLVDYKDDDDKRS

SEQ ID NO: 127 - DNA, 16 bp, synthetic construct
  misc_feature 1..16: note = AAV-ITR-Forward Primer
  source 1..16: mol_type = other DNA
cggcctcagtgagcga

SEQ ID NO: 128 - DNA, 21 bp, synthetic construct
  misc_feature 1..21: note = AAV-ITR-Reverse primer
  source 1..21: mol_type = other DNA
ggaacccctagtgatggagtt

SEQ ID NO: 129 - DNA, 19 bp, synthetic construct
  misc_feature 1..19: note = gRNA spacer sequence
  source 1..19: mol_type = other DNA
acagtgggcaggattgaaa

SEQ ID NO: 130 - DNA, 19 bp, synthetic construct
  misc_feature 1..19: note = gRNA spacer sequence
  source 1..19: mol_type = other DNA
gcaggtgcactcaccgggt

SEQ ID NO: 131 - DNA, 20 bp, synthetic construct
  misc_feature 1..20: note = gRNA spacer sequence
  source 1..20: mol_type = other DNA
gagctcagggagcatcgagg

SEQ ID NO: 132 - DNA, 19 bp, synthetic construct
  misc_feature 1..19: note = gRNA spacer sequence
  source 1..19: mol_type = other DNA
agagtcgcaattggagcgc

SEQ ID NO: 133 - DNA, 19 bp, synthetic construct
  misc_feature 1..19: note = gFNA spacer sequence
  source 1..19: mol_type = other DNA
ccagaccagcctgcacagt

SEQ ID NO: 134 - DNA, 20 bp, synthetic construct
  misc_feature 1..20: note = gRNA spacer sequence
  source 1..20: mol_type = other DNA
gagcgcaggctaggcctgca

SEQ ID NO: 135 - DNA, 19 bp, synthetic construct
  misc_feature 1..19: note = gRNA spacer sequence
  source 1..19: mol_type = other DNA
ctaggagtccgggataccc

SEQ ID NO: 136 - DNA, 20 bp, synthetic construct
  misc_feature 1..20: note = gRNA spacer sequence
  source 1..20: mol_type = other DNA
gaatccgcaggtgcactcac

SEQ ID NO: 137 - DNA, 20 bp, synthetic construct
  misc_feature 1..20: note = gRNA spacer sequence
  source 1..20: mol_type = other DNA
gaccagcctgcacagtgggc

SEQ ID NO: 138 - DNA, 20 bp, synthetic construct
  misc_feature 1..20: note = gRNA spacer sequence
  source 1..20: mol_type = other DNA
gcgacgcggttggcagccga

SEQ ID NO: 139 - DNA, 18 bp, synthetic construct
  misc_feature 1..18: note = ZF target sequence
  source 1..18: mol_type = other DNA
ggcgaggtgatggaaggg

SEQ ID NO: 140 - DNA, 18 bp, synthetic construct
  misc_feature 1..18: note = ZF target sequence
  source 1..18: mol_type = other DNA
gagggagctaggggtggg

SEQ ID NO: 141 - DNA, 18 bp, synthetic construct
  misc_feature 1..18: note = ZF target sequence
  source 1..18: mol_type = other DNA
agtgctaatgtttccgag

SEQ ID NO: 142 - DNA, 18 bp, synthetic construct
  misc_feature 1..18: note = ZF target sequence
  source 1..18: mol_type = other DNA
tagacggtgcagggcgga

SEQ ID NO: 143 - protein, 25 aa, synthetic construct
  REGION 1..25: note = ZF binding domain consensus sequence
  REGION 2..5: note = MISC_FEATURE - X is any amino acid and wherein positions 2 and 3 may be present or absent
  REGION 7..18: note = MISC_FEATURE - X is any amino acid
  REGION 20..24: note = MISC_FEATURE - X is any amino acid
CXXXXCXXXXXXXXXXXXHXXXXXH